European Patent Application EP 4 595 979 A1, published August 6, 2025. Title: AURISTATIN DRUG WITH HIGH-STABILITY HYDROPHILIC LINKING UNIT AND CONJUGATE THEREOF. Applicant: SYSTIMMUNE, INC. Application EP 23870979.4, filed September 28, 2023. The sequence listing filed with the application follows.

SEQUENCE LISTING (54 sequences)

SEQ ID NO: 1 - protein, 11 aa, synthetic construct
RASQDINKYLA

SEQ ID NO: 2 - protein, 7 aa, synthetic construct
STSTLQS

SEQ ID NO: 3 - protein, 8 aa, synthetic construct
LQYDDLFT

SEQ ID NO: 4 - protein, 5 aa, synthetic construct
SFDIN

SEQ ID NO: 5 - protein, 17 aa, synthetic construct
WIFPGDGNTKYSQKFQG

SEQ ID NO: 6 - protein, 9 aa, synthetic construct
GEALYYFDY

SEQ ID NO: 7 - protein, 106 aa, synthetic construct
DIQMTQSPSSLSASVGDRVTITCRASQDINKYLAWYQQKPGKVPKLLIYSTSTLQSGVPSRFSGSGSGTDFTLTISSLQPEDVATYYCLQYDDLFTFGQGTKLEIK

SEQ ID NO: 8 - protein, 107 aa, synthetic construct [sequence omitted]

SEQ ID NO: 9 - protein, 213 aa, synthetic construct
DIQMTQSPSSLSASVGDRVTITCRASQDINKYLAWYQQKPGKVPKLLIYSTSTLQSGVPSRFSGSGSGTDFTLTISSLQPEDVATYYCLQYDDLFTFGQGTKLEIKRTVAAPSVFIFPPSDEQLKSGTASVVCLLNNFYPREAKVQWKVDNALQSGNSQESVTEQDSKDSTYSLSSTLTLSKADYEKHKVYACEVTHQGLSSPVTKSFNRGEC

SEQ ID NO: 10 - protein, 106 aa, synthetic construct; identical to SEQ ID NO: 7

SEQ ID NO: 11 - protein, 108 aa, synthetic construct
RTVAAPSVFIFPPSDEQLKSGTASVVCLLNNFYPREAKVQWKVDNALQSGNSQESVTEQDSKDSTYSLSSTLTLSKADYEKHKVYACEVTHQGLSSPVCTKSFNRGEC

SEQ ID NO: 12 - protein, 214 aa, synthetic construct
DIQMTQSPSSLSASVGDRVTITCRASQDINKYLAWYQQKPGKVPKLLIYSTSTLQSGVPSRFSGSGSGTDFTLTISSLQPEDVATYYCLQYDDLFTFGQGTKLEIKRTVAAPSVFIFPPSDEQLKSGTASVVCLLNNFYPREAKVQWKVDNALQSGNSQESVTEQDSKDSTYSLSSTLTLSKADYEKHKVYACEVTHQGLSSPVCTKSFNRGEC

SEQ ID NO: 13 - protein, 118 aa, synthetic construct
QVQLVQSGAEVKKPGASVKLSCKASGYTFTSFDINWVRQAPEQRLEWMGWIFPGDGNTKYSQKFQGRATITRDTSASTAYMELSSLRSEDTAVYYCVRGEALYYFDYWGQGTLVTVSS

SEQ ID NO: 14 - protein, 329 aa, synthetic construct
ASTKGPSVFPLAPSSKSTSGGTAALGCLVKDYFPEPVTVSWNSGALTSGVHTFPAVLQSSGLYSLSSVVTVPSSSLGTQTYICNVNHKPSNTKVDKRVEPKSCDKTHTCPPCPAPELLGGPSVFLFPPKPKDTLMISRTPEVTCVVVDVSHEDPEVKFNWYVDGVEVHNAKTKPREEQYNSTYRVVSVLTVLHQDWLNGKEYKCKVSNKALPAPIEKTISKAKGQPREPQVYTLPPSRDELTKNQVSLTCLVKGFYPSDIAVEWESNGQPENNYKTTPPVLDSDGSFFLYSKLTVDKSRWQQGNVFSCSVMHEALHNHYTQKSLSLSPG

SEQ ID NO: 15 - protein, 447 aa, synthetic construct
QVQLVQSGAEVKKPGASVKLSCKASGYTFTSFDINWVRQAPEQRLEWMGWIFPGDGNTKYSQKFQGRATITRDTSASTAYMELSSLRSEDTAVYYCVRGEALYYFDYWGQGTLVTVSSASTKGPSVFPLAPSSKSTSGGTAALGCLVKDYFPEPVTVSWNSGALTSGVHTFPAVLQSSGLYSLSSVVTVPSSSLGTQTYICNVNHKPSNTKVDKRVEPKSCDKTHTCPPCPAPELLGGPSVFLFPPKPKDTLMISRTPEVTCVVVDVSHEDPEVKFNWYVDGVEVHNAKTKPREEQYNSTYRVVSVLTVLHQDWLNGKEYKCKVSNKALPAPIEKTISKAKGQPREPQVYTLPPSRDELTKNQVSLTCLVKGFYPSDIAVEWESNGQPENNYKTTPPVLDSDGSFFLYSKLTVDKSRWQQGNVFSCSVMHEALHNHYTQKSLSLSPG

SEQ ID NO: 16 - DNA, 33 bp, synthetic construct
  source 1..33: mol_type = other DNA
agagcttctcaggatatcaataagtatctggct

SEQ ID NO: 17 - DNA, 21 bp, synthetic construct
  source 1..21: mol_type = other DNA
tctacatctaccctgcagtct

SEQ ID NO: 18 - DNA, 24 bp, synthetic construct
  source 1..24: mol_type = other DNA
ctgcagtatgatgatctgttcacc

SEQ ID NO: 19 - DNA, 15 bp, synthetic construct
  source 1..15: mol_type = other DNA
tccttcgacattaac

SEQ ID NO: 20 - DNA, 51 bp, synthetic construct
  source 1..51: mol_type = other DNA
tggatcttccccggcgacggcaacaccaagtactcccagaagttccaggga

SEQ ID NO: 21 - DNA, 27 bp, synthetic construct
  source 1..27: mol_type = other DNA
ggagaggctctgtactattttgattat

SEQ ID NO: 22 - DNA, 318 bp, synthetic construct
  source 1..318: mol_type = other DNA
gatatccagatgacccagtctccatctagcctgtccgcttctgtgggcgatagagtgaccatcacatgcagagcttctcaggatatcaataagtatctggcttggtatcagcagaagcctggaaaggtgcctaagctgctgatctactctacatctaccctgcagtctggagtgccttctagattttctggatctggctctggcaccgattttacactgacaatctcttctctgcagcctgaggatgtggctacatattattgtctgcagtatgatgatctgttcacctttggccagggcaccaagctggagatcaag

SEQ ID NO: 23 - DNA, 324 bp, synthetic construct
  source 1..324: mol_type = other DNA
cgtacggtggctgcaccatctgtcttcatcttcccgccatctgatgagcagttgaaatctggaactgcctctgttgtgtgcctgctgaataacttctatcccagagaggccaaagtacagtggaaggtggataacgccctccaatcgggtaactcccaggagagtgtcacagagcaggacagcaaggacagcacctacagcctcagcagcaccctgacgctgagcaaagcagactacgagaaacacaaagtctacgcctgcgaagtcacccatcagggcctgagctcgcccgtcacaaagagcttcaacaggggagagtgttag

SEQ ID NO: 24 - DNA, 642 bp, synthetic construct
  source 1..642: mol_type = other DNA
gatatccagatgacccagtctccatctagcctgtccgcttctgtgggcgatagagtgaccatcacatgcagagcttctcaggatatcaataagtatctggcttggtatcagcagaagcctggaaaggtgcctaagctgctgatctactctacatctaccctgcagtctggagtgccttctagattttctggatctggctctggcaccgattttacactgacaatctcttctctgcagcctgaggatgtggctacatattattgtctgcagtatgatgatctgttcacctttggccagggcaccaagctggagatcaagcgtacggtggctgcaccatctgtcttcatcttcccgccatctgatgagcagttgaaatctggaactgcctctgttgtgtgcctgctgaataacttctatcccagagaggccaaagtacagtggaaggtggataacgccctccaatcgggtaactcccaggagagtgtcacagagcaggacagcaaggacagcacctacagcctcagcagcaccctgacgctgagcaaagcagactacgagaaacacaaagtctacgcctgcgaagtcacccatcagggcctgagctcgcccgtcacaaagagcttcaacaggggagagtgttag

SEQ ID NO: 25 - DNA, 318 bp, synthetic construct; identical to SEQ ID NO: 22
  source 1..318: mol_type = other DNA

SEQ ID NO: 26 - DNA, 327 bp, synthetic construct
  source 1..327: mol_type = other DNA
cgtacggtggctgcaccatctgtcttcatcttcccgccatctgatgagcagttgaaatctggaactgcctctgttgtgtgcctgctgaataacttctatcccagagaggccaaagtacagtggaaggtggataacgccctccaatcgggtaactcccaggagagtgtcacagagcaggacagcaaggacagcacctacagcctcagcagcaccctgacgctgagcaaagcagactacgagaaacacaaagtctacgcctgcgaagtcacccatcagggcctgagctcgcccgtctgtacaaagagcttcaacaggggagagtgttag

SEQ ID NO: 27 - DNA, 645 bp, synthetic construct
  source 1..645: mol_type = other DNA
gatatccagatgacccagtctccatctagcctgtccgcttctgtgggcgatagagtgaccatcacatgcagagcttctcaggatatcaataagtatctggcttggtatcagcagaagcctggaaaggtgcctaagctgctgatctactctacatctaccctgcagtctggagtgccttctagattttctggatctggctctggcaccgattttacactgacaatctcttctctgcagcctgaggatgtggctacatattattgtctgcagtatgatgatctgttcacctttggccagggcaccaagctggagatcaagcgtacggtggctgcaccatctgtcttcatcttcccgccatctgatgagcagttgaaatctggaactgcctctgttgtgtgcctgctgaataacttctatcccagagaggccaaagtacagtggaaggtggataacgccctccaatcgggtaactcccaggagagtgtcacagagcaggacagcaaggacagcacctacagcctcagcagcaccctgacgctgagcaaagcagactacgagaaacacaaagtctacgcctgcgaagtcacccatcagggcctgagctcgcccgtctgtacaaagagcttcaacaggggagagtgttag

SEQ ID NO: 28 - DNA, 354 bp, synthetic construct
  source 1..354: mol_type = other DNA
caggtgcagctggtgcagtccggcgccgaggtgaagaagcccggcgcctccgtgaagctgagctgtaaggcctccggctacaccttcacctccttcgacattaactgggtgcggcaggcccccgagcagcgcctggagtggatgggctggatcttccccggcgacggcaacaccaagtactcccagaagttccagggaagagctaccatcaccagagatacatccgcttctacagcttacatggagctgtctagcctgagatctgaggatacagctgtgtattactgtgtgagaggagaggctctgtactattttgattattggggccagggcaccctggtgacagtgtcttct

SEQ ID NO: 29 - DNA, 990 bp, synthetic construct
  source 1..990: mol_type = other DNA
gctagcaccaagggcccatcggtcttccccctggcaccctcctccaagagcacctctgggggcacagcggccctgggctgcctggtcaaggactacttccccgaaccggtgacggtgtcgtggaactcaggcgccctgaccagcggcgtgcacaccttcccggctgtcctacagtcctcaggactctactccctcagcagcgtggtgaccgtgccctccagcagcttgggcacccagacctacatctgcaacgtgaatcacaagcccagcaacaccaaggtggacaagagagttgagcccaaatcttgtgacaaaactcacacatgcccaccgtgcccagcacctgaactcctggggggaccgtcagtcttcctcttccccccaaaacccaaggacaccctcatgatctcccggacccctgaggtcacatgcgtggtggtggacgtgagccacgaagaccctgaggtcaagttcaactggtacgtggacggcgtggaggtgcataatgccaagacaaagccgcgggaggagcagtacaacagcacgtaccgtgtggtcagcgtcctcaccgtcctgcaccaggactggctgaatggcaaggagtacaagtgcaaggtctccaacaaagccctcccagcccccatcgagaaaaccatctccaaagccaaagggcagccccgagaaccacaggtgtacaccctgcccccatcccgggatgagctgaccaagaaccaggtcagcctgacctgcctggtcaaaggcttctatcccagcgacatcgccgtggagtgggagagcaatgggcagccggagaacaactacaagaccacgcctcccgtgctggactccgacggctccttcttcctctatagcaagctcaccgtggacaagagcaggtggcagcaggggaacgtcttctcatgctccgtgatgcatgaggctctgcacaaccactacacgcagaagagcctctccctgtctccgggttaa

SEQ ID NO: 30 - DNA, 1344 bp, synthetic construct
  source 1..1344: mol_type = other DNA
caggtgcagctggtgcagtccggcgccgaggtgaagaagcccggcgcctccgtgaagctgagctgtaaggcctccggctacaccttcacctccttcgacattaactgggtgcggcaggcccccgagcagcgcctggagtggatgggctggatcttccccggcgacggcaacaccaagtactcccagaagttccagggaagagctaccatcaccagagatacatccgcttctacagcttacatggagctgtctagcctgagatctgaggatacagctgtgtattactgtgtgagaggagaggctctgtactattttgattattggggccagggcaccctggtgacagtgtcttctgctagcaccaagggcccatcggtcttccccctggcaccctcctccaagagcacctctgggggcacagcggccctgggctgcctggtcaaggactacttccccgaaccggtgacggtgtcgtggaactcaggcgccctgaccagcggcgtgcacaccttcccggctgtcctacagtcctcaggactctactccctcagcagcgtggtgaccgtgccctccagcagcttgggcacccagacctacatctgcaacgtgaatcacaagcccagcaacaccaaggtggacaagagagttgagcccaaatcttgtgacaaaactcacacatgcccaccgtgcccagcacctgaactcctggggggaccgtcagtcttcctcttccccccaaaacccaaggacaccctcatgatctcccggacccctgaggtcacatgcgtggtggtggacgtgagccacgaagaccctgaggtcaagttcaactggtacgtggacggcgtggaggtgcataatgccaagacaaagccgcgggaggagcagtacaacagcacgtaccgtgtggtcagcgtcctcaccgtcctgcaccaggactggctgaatggcaaggagtacaagtgcaaggtctccaacaaagccctcccagcccccatcgagaaaaccatctccaaagccaaagggcagccccgagaaccacaggtgtacaccctgcccccatcccgggatgagctgaccaagaaccaggtcagcctgacctgcctggtcaaaggcttctatcccagcgacatcgccgtggagtgggagagcaatgggcagccggagaacaactacaagaccacgcctcccgtgctggactccgacggctccttcttcctctatagcaagctcaccgtggacaagagcaggtggcagcaggggaacgtcttctcatgctccgtgatgcatgaggctctgcacaaccactacacgcagaagagcctctccctgtctccgggttaa

SEQ ID NO: 31 - protein, 11 aa, synthetic construct
KASQSVSNDVV

SEQ ID NO: 32 - protein, 7 aa, synthetic construct
YASNRYT

SEQ ID NO: 33 - protein, 9 aa, synthetic construct
QQDYSSPWT

SEQ ID NO: 34 - protein, 5 aa, synthetic construct
DHVIS

SEQ ID NO: 35 - protein, 17 aa, synthetic construct
QIYPGSDNSYYAQKFQG

SEQ ID NO: 36 - protein, 16 aa, synthetic construct
EGYGYGKNGVGYAMDY

SEQ ID NO: 37 - protein, 107 aa, synthetic construct
DIVMTQSPDSLAVSLGERATINCKASQSVSNDVVWYQQKPGQPPKLLIYYASNRYTGVPDRFSGSGYGTDFTLTISSLQAEDVAVYYCQQDYSSPWTFGGGTKVEIK

SEQ ID NO: 38 - protein, 107 aa, synthetic construct [sequence omitted]

SEQ ID NO: 39 - protein, 214 aa, synthetic construct
DIVMTQSPDSLAVSLGERATINCKASQSVSNDVVWYQQKPGQPPKLLIYYASNRYTGVPDRFSGSGYGTDFTLTISSLQAEDVAVYYCQQDYSSPWTFGGGTKVEIKRTVAAPSVFIFPPSDEQLKSGTASVVCLLNNFYPREAKVQWKVDNALQSGNSQESVTEQDSKDSTYSLSSTLTLSKADYEKHKVYACEVTHQGLSSPVTKSFNRGEC

SEQ ID NO: 40 - protein, 125 aa, synthetic construct
QVQLVQSGAEVKKPGASVKVSCKASGYTFTDHVISWVRQATGQGLEWMGQIYPGSDNSYYAQKFQGRVTLTADKSINTAYMELSSLRSEDTAVYYCAREGYGYGKNGVGYAMDYWGQGTLVTVSS

SEQ ID NO: 41 - protein, 329 aa, synthetic construct; identical to SEQ ID NO: 14

SEQ ID NO: 42 - protein, 454 aa, synthetic construct
QVQLVQSGAEVKKPGASVKVSCKASGYTFTDHVISWVRQATGQGLEWMGQIYPGSDNSYYAQKFQGRVTLTADKSINTAYMELSSLRSEDTAVYYCAREGYGYGKNGVGYAMDYWGQGTLVTVSSASTKGPSVFPLAPSSKSTSGGTAALGCLVKDYFPEPVTVSWNSGALTSGVHTFPAVLQSSGLYSLSSVVTVPSSSLGTQTYICNVNHKPSNTKVDKRVEPKSCDKTHTCPPCPAPELLGGPSVFLFPPKPKDTLMISRTPEVTCVVVDVSHEDPEVKFNWYVDGVEVHNAKTKPREEQYNSTYRVVSVLTVLHQDWLNGKEYKCKVSNKALPAPIEKTISKAKGQPREPQVYTLPPSRDELTKNQVSLTCLVKGFYPSDIAVEWESNGQPENNYKTTPPVLDSDGSFFLYSKLTVDKSRWQQGNVFSCSVMHEALHNHYTQKSLSLSPG

SEQ ID NO: 43 - DNA, 33 bp, synthetic construct
  source 1..33: mol_type = other DNA
aaggcttctcagtctgtgtctaatgatgtggtg

SEQ ID NO: 44 - DNA, 21 bp, synthetic construct
  source 1..21: mol_type = other DNA
tacgcctccaacaggtacacc

SEQ ID NO: 45 - DNA, 27 bp, synthetic construct
  source 1..27: mol_type = other DNA
cagcaggactactcctccccctggacc

SEQ ID NO: 46 - DNA, 15 bp, synthetic construct
  source 1..15: mol_type = other DNA
gaccacgtgatctcc

SEQ ID NO: 47 - DNA, 51 bp, synthetic construct
  source 1..51: mol_type = other DNA
cagatctaccccggctccgacaactcctactacgcccagaagttccagggc

SEQ ID NO: 48 - DNA, 48 bp, synthetic construct
  source 1..48: mol_type = other DNA
gagggctacggctacggcaagaacggcgtgggctacgccatggattat

SEQ ID NO: 49 - DNA, 321 bp, synthetic construct
  source 1..321: mol_type = other DNA
gatatcgtgatgacacagtctcctgattctctggccgtgtctctgggcgaaagagctacaatcaactgtaaggcttctcagtctgtgtctaatgatgtggtgtggtaccagcagaagcctgggcagccccccaagctgctgatctactacgcctccaacaggtacaccggcgtgcccgacaggttctccggctccggctacggcaccgacttcaccctgaccatctcctccctgcaggccgaggacgtggccgtgtactactgccagcaggactactcctccccctggaccttcggcggcggcaccaaggtggagatcaag

SEQ ID NO: 50 - DNA, 324 bp, synthetic construct; identical to SEQ ID NO: 23
  source 1..324: mol_type = other DNA

SEQ ID NO: 51 - DNA, 645 bp, synthetic construct
  source 1..645: mol_type = other DNA
gatatcgtgatgacacagtctcctgattctctggccgtgtctctgggcgaaagagctacaatcaactgtaaggcttctcagtctgtgtctaatgatgtggtgtggtaccagcagaagcctgggcagccccccaagctgctgatctactacgcctccaacaggtacaccggcgtgcccgacaggttctccggctccggctacggcaccgacttcaccctgaccatctcctccctgcaggccgaggacgtggccgtgtactactgccagcaggactactcctccccctggaccttcggcggcggcaccaaggtggagatcaagcgtacggtggctgcaccatctgtcttcatcttcccgccatctgatgagcagttgaaatctggaactgcctctgttgtgtgcctgctgaataacttctatcccagagaggccaaagtacagtggaaggtggataacgccctccaatcgggtaactcccaggagagtgtcacagagcaggacagcaaggacagcacctacagcctcagcagcaccctgacgctgagcaaagcagactacgagaaacacaaagtctacgcctgcgaagtcacccatcagggcctgagctcgcccgtcacaaagagcttcaacaggggagagtgttag

SEQ ID NO: 52 - DNA, 375 bp, synthetic construct
  source 1..375: mol_type = other DNA
caggtgcagctggtgcagtctggggccgaggtgaaaaagccaggcgcttctgtgaaggtgtcttgcaaggcctccggctacaccttcaccgaccacgtgatctcctgggtgcgccaggccaccggccagggcctggagtggatgggccagatctaccccggctccgacaactcctactacgcccagaagttccagggcagggtgactctgaccgccgacaagtccatcaacaccgcctacatggagctgtcctccctgaggtccgaggacaccgccgtgtactactgcgccagggagggctacggctacggcaagaacggcgtgggctacgccatggattattggggccagggcaccctggtgacagtgtcttct

SEQ ID NO: 53 - DNA, 990 bp, synthetic construct; identical to SEQ ID NO: 29
  source 1..990: mol_type = other DNA

SEQ ID NO: 54 - DNA, 1365 bp, synthetic construct
  source 1..1365: mol_type = other DNA
caggtgcagctggtgcagtctggggccgaggtgaaaaagccaggcgcttctgtgaaggtgtcttgcaaggcctccggctacaccttcaccgaccacgtgatctcctgggtgcgccaggccaccggccagggcctggagtggatgggccagatctaccccggctccgacaactcctactacgcccagaagttccagggcagggtgactctgaccgccgacaagtccatcaacaccgcctacatggagctgtcctccctgaggtccgaggacaccgccgtgtactactgcgccagggagggctacggctacggcaagaacggcgtgggctacgccatggattattggggccagggcaccctggtgacagtgtcttctgctagcaccaagggcccatcggtcttccccctggcaccctcctccaagagcacctctgggggcacagcggccctgggctgcctggtcaaggactacttccccgaaccggtgacggtgtcgtggaactcaggcgccctgaccagcggcgtgcacaccttcccggctgtcctacagtcctcaggactctactccctcagcagcgtggtgaccgtgccctccagcagcttgggcacccagacctacatctgcaacgtgaatcacaagcccagcaacaccaaggtggacaagagagttgagcccaaatcttgtgacaaaactcacacatgcccaccgtgcccagcacctgaactcctggggggaccgtcagtcttcctcttccccccaaaacccaaggacaccctcatgatctcccggacccctgaggtcacatgcgtggtggtggacgtgagccacgaagaccctgaggtcaagttcaactggtacgtggacggcgtggaggtgcataatgccaagacaaagccgcgggaggagcagtacaacagcacgtaccgtgtggtcagcgtcctcaccgtcctgcaccaggactggctgaatggcaaggagtacaagtgcaaggtctccaacaaagccctcccagcccccatcgagaaaaccatctccaaagccaaagggcagccccgagaaccacaggtgtacaccctgcccccatcccgggatgagctgaccaagaaccaggtcagcctgacctgcctggtcaaaggcttctatcccagcgacatcgccgtggagtgggagagcaatgggcagccggagaacaactacaagaccacgcctcccgtgctggactccgacggctccttcttcctctatagcaagctcaccgtggacaagagcaggtggcagcaggggaacgtcttctcatgctccgtgatgcatgaggctctgcacaaccactacacgcagaagagcctctccctgtctccgggttaa